European Patent Specification EP 3 708 667 B1, published January 1, 2025. Title: IMMUNOGLOBULIN-BINDING PROTEIN. Applicant: TOSOH Corporation. The sequence listing filed with the application follows.

SEQUENCE LISTING (40 sequences)

SEQ ID NO: 1 - protein, 58 aa, Staphylococcus aureus
ADNKFNKEQQNAFYEILHLPNLTEEQRNGFIQSLKDDPSVSKEILAEAKKLNDAQAPK

SEQ ID NO: 2 - protein, 58 aa, Artificial Sequence
  Lys49Met
ADNKFNKEQQNAFYEILHLPNLTEEQRNGFIQSLKDDPSVSKEILAEAMKLNDAQAPK

SEQ ID NO: 3 - DNA, 174 bp, Artificial Sequence
  E.coli codon
gcggataacaagttcaacaaagaacagcagaatgccttttatgagattctgcatttaccgaatctgaccgaagaacaacgcaatggctttatccagtcgttgaaagacgatccaagtgtgagcaaagagattctggcagaagccaagaaactcaacgatgcgcaagctccgaaa

SEQ ID NO: 4 - DNA, 26 bp, Artificial Sequence
  Oligonucleotide
tagccatgggcgcggataacaagttc

SEQ ID NO: 5 - DNA, 27 bp, Artificial Sequence
  Oligonucleotide
ctactcgagtttcggagcttgcgcatc

SEQ ID NO: 6 - DNA, 20 bp, Artificial Sequence
  Oligonucleotide
taatacgactcactataggg

SEQ ID NO: 7 - DNA, 19 bp, Artificial Sequence
  Oligonucleotide
tatgctagttattgctcag

SEQ ID NO: 8 - protein, 58 aa, Artificial Sequence
  SpA1(Asn21Tyr)
ADNKFNKEQQNAFYEILHLPYLTEEQRNGFIQSLKDDPSVSKEILAEAKKLNDAQAPK

SEQ ID NO: 9 - protein, 58 aa, Artificial Sequence
  Lys58Glu
ADNKFNKEQQNAFYEILHLPNLTEEQRNGFIQSLKDDPSVSKEILAEAKKLNDAQAPE

SEQ ID NO: 10 - DNA, 174 bp, Artificial Sequence
  Polynucleotide encoding SpA1
gcggataacaagttcaacaaagaacagcagaatgccttttatgagattctgcatttaccgtatctgaccgaagaacaacgcaatggctttatccagtcgttgaaagacgatccaagtgtgagcaaagagattctggcagaagccaagaaactcaacgatgcgcaagctccgaaa

SEQ ID NO: 11 - protein, 58 aa, Artificial Sequence
  SpA'(Gly29Ala)
ADNKFNKEQQNAFYEILHLPNLTEEQRNAFIQSLKDDPSVSKEILAEAKKLNDAQAPK

SEQ ID NO: 12 - DNA, 174 bp, Artificial Sequence
  Polynucleotide encoding SpA'
gcggataacaagttcaacaaagaacagcagaatgccttttatgagattctgcatttaccgaatctgaccgaagaacaacgcaatgcctttatccagtcgttgaaagacgatccaagtgtgagcaaagagattctggcagaagccaagaaactcaacgatgcgcaagctccgaaa

SEQ ID NO: 13 - protein, 58 aa, Artificial Sequence
  SpA2(Lys7Glu,Asn21Tyr,Gly29Ala)
ADNKFNEEQQNAFYEILHLPYLTEEQRNAFIQSLKDDPSVSKEILAEAKKLNDAQAPK

SEQ ID NO: 14 - DNA, 174 bp, Artificial Sequence
  Polynucleotide encoding SpA2
gcggacaacaaattcaacgaagaacagcagaatgccttttacgagattctgcatttaccgtatctgaccgaagaacaacgcaatgcctttatccagagcttgaaagatgatccgagtgtgtcgaaagagattctcgctgaagcgaagaaactgaacgatgcacaagcgccaaaa

SEQ ID NO: 15 - protein, 58 aa, Artificial Sequence
  SpA3a(Lys7Glu,Asn21Tyr,Gly29Ala,Lys58Glu)
ADNKFNEEQQNAFYEILHLPYLTEEQRNAFIQSLKDDPSVSKEILAEAKKLNDAQAPE

SEQ ID NO: 16 - DNA, 174 bp, Artificial Sequence
  Polynucleotide encoding SpA3a
gcggacaacaaattcaacgaagaacagcagaatgccttttacgagattctgcatttaccgtatctgaccgaagaacaacgcaatgcctttatccagagcttgaaagatgatccgagtgtgtcgaaagagattctcgctgaagcgaagaaactgaacgatgcacaagcgccagaa

SEQ ID NO: 17 - protein, 58 aa, Artificial Sequence
  SpA4a(Lys4Arg,Lys7Glu,Asn21Tyr,Gly29Ala,Lys58Glu)
ADNRFNEEQQNAFYEILHLPYLTEEQRNAFIQSLKDDPSVSKEILAEAKKLNDAQAPE

SEQ ID NO: 18 - DNA, 174 bp, Artificial Sequence
  Polynucleotide encoding SpA4a
gcggacaatcgattcaacgaagaacagcagaatgccttttacgagattctgcatttaccgtatctgaccgaagaacaacgcaatgcctttatccagagcttgaaagatgatccgagtgtgtcgaaagagattctcgctgaagcgaagaaactgaacgatgcacaagcgccagaa

SEQ ID NO: 19 - protein, 58 aa, Artificial Sequence
  SpA5a(Lys4Arg,Lys7Glu,Asn21Tyr,Gly29Ala,Lys49Met,Lys58Glu)
ADNRFNEEQQNAFYEILHLPYLTEEQRNAFIQSLKDDPSVSKEILAEAMKLNDAQAPE

SEQ ID NO: 20 - DNA, 174 bp, Artificial Sequence
  Polynucleotide encoding SpA5a
gcggacaaccgcttcaacgaagaacagcagaatgccttttacgagattctgcatttaccgtatctgaccgaagaacaacgcaatgcctttatccagagcttgaaagatgatccgagtgtgtcgaaagagattctcgctgaagcgatgaaactgaacgatgcacaagcgccagaa

SEQ ID NO: 21 - protein, 58 aa, Artificial Sequence
  SpA3b(Lys4Arg,Lys7Glu,Gly29Ala,Lys58Glu)
ADNRFNEEQQNAFYEILHLPNLTEEQRNAFIQSLKDDPSVSKEILAEAKKLNDAQAPE

SEQ ID NO: 22 - DNA, 174 bp, Artificial Sequence
  Polynucleotide encoding SpA3b
gcggacaaccgcttcaacgaagaacagcagaatgccttttacgagattctgcatttaccgaatctgaccgaagaacaacgcaatgcctttatccagagcttgaaagatgatccgagtgtgtcgaaagagattctcgctgaagcgaagaaactgaacgatgcacaagcgccagaa

SEQ ID NO: 23 - DNA, 23 bp, Artificial Sequence
  Oligonucleotide
tagccatgggcgcggacaacaaa

SEQ ID NO: 24 - DNA, 26 bp, Artificial Sequence
  Oligonucleotide
tagccatgggcgcggacaatcgattc

SEQ ID NO: 25 - DNA, 32 bp, Artificial Sequence
  Oligonucleotide
tagccatgggcgcggacaaccgcttcaacgaa

SEQ ID NO: 26 - DNA, 27 bp, Artificial Sequence
  Oligonucleotide
ctactcgagttttggcgcttgtgcatc

SEQ ID NO: 27 - DNA, 33 bp, Artificial Sequence
  Oligonucleotide
ctactcgagttctggcgcttgtgcatcgttcag

SEQ ID NO: 28 - protein, 58 aa, Artificial Sequence
  SpA5b(Asn3Ile,Lys4Arg,Lys7Glu,Asn21Tyr,Gly29Ala,Lys58Glu)
ADIRFNEEQQNAFYEILHLPYLTEEQRNAFIQSLKDDPSVSKEILAEAKKLNDAQAPE

SEQ ID NO: 29 - protein, 58 aa, Artificial Sequence
  SpA5c(Asn3Thr,Lys4Arg,Lys7Glu,Asn21Tyr,Gly29Ala,Lys58Glu)
ADTRFNEEQQNAFYEILHLPYLTEEQRNAFIQSLKDDPSVSKEILAEAKKLNDAQAPE

SEQ ID NO: 30 - protein, 58 aa, Artificial Sequence
  SpA5d(Lys4Arg,Lys7Glu,Asn11Lys,Asn21Tyr,Gly29Ala,Lys58Glu)
ADNRFNEEQQKAFYEILHLPYLTEEQRNAFIQSLKDDPSVSKEILAEAKKLNDAQAPE

SEQ ID NO: 31 - protein, 58 aa, Artificial Sequence
  SpA5e(Lys4Arg,Lys7Glu,Asn11Tyr,Asn21Tyr,Gly29Ala,Lys58Glu)
ADNRFNEEQQYAFYEILHLPYLTEEQRNAFIQSLKDDPSVSKEILAEAKKLNDAQAPE

SEQ ID NO: 32 - protein, 58 aa, Artificial Sequence
  SpA4b(Lys4Arg,Lys7Glu,Asn21Tyr,Gly29Ala,Lys58Val)
ADNRFNEEQQNAFYEILHLPYLTEEQRNAFIQSLKDDPSVSKEILAEAKKLNDAQAPV

SEQ ID NO: 33 - DNA, 174 bp, Artificial Sequence
  Polynucleotide encoding SpA5d
gcggacaatcgattcaacgaagaacagcagaaagccttttacgagattctgcatttaccgtatctgaccgaagaacaacgcaatgcctttatccagagcttgaaagatgatccgagtgtgtcgaaagagattctcgctgaagcgaagaaactgaacgatgcacaagcgccagaa

SEQ ID NO: 34 - protein, 58 aa, Artificial Sequence
  SpA6a(Lys4Arg,Lys7Glu,Asn11Lys,Glu15Ala,Asn21Tyr,Gly29Ala,Lys58Gl u)
ADNRFNEEQQKAFYAILHLPYLTEEQRNAFIQSLKDDPSVSKEILAEAKKLNDAQAPE

SEQ ID NO: 35 - protein, 58 aa, Artificial Sequence
  SpA5f(Lys4Arg,Lys7Glu,Asn11Lys,Asn21Tyr,Gly29Ala,Lys58Gly)
ADNRFNEEQQKAFYEILHLPYLTEEQRNAFIQSLKDDPSVSKEILAEAKKLNDAQAPG

SEQ ID NO: 36 - DNA, 174 bp, Artificial Sequence
  Polynucleotide encoding SpA6a
gcggacaatcgattcaacgaagaacagcagaaagccttttacgcgattctgcatttaccgtatctgactgaagaacaacgcaatgcctttatccagagcttgaaagatgatccgagtgtgtcgaaagagattctcgctgaagcgaagaaactgaacgatgcacaagcgccagaa

SEQ ID NO: 37 - protein, 58 aa, Artificial Sequence
  SpA7a(Lys4Arg,Lys7Glu,Asn11Lys,Glu15Ala,Asn21Tyr,Gly29Ala,Val40Al a,Lys58Glu)
ADNRFNEEQQKAFYAILHLPYLTEEQRNAFIQSLKDDPSASKEILAEAKKLNDAQAPE

SEQ ID NO: 38 - protein, 58 aa, Artificial Sequence
  SpA7b(Asn3Ile,Lys4Arg,Lys7Glu,Asn11Lys,Glu15Ala,Asn21Tyr,Gly29Ala ,Lys58Glu)
ADIRFNEEQQKAFYAILHLPYLTEEQRNAFIQSLKDDPSVSKEILAEAKKLNDAQAPE

SEQ ID NO: 39 - protein, 58 aa, Artificial Sequence
  SpA6b(Lys4Arg,Lys7Glu,Asn11Lys,Glu15Ala,Asn21Tyr,Gly29Ala,Lys58As p)
ADNRFNEEQQKAFYAILHLPYLTEEQRNAFIQSLKDDPSVSKEILAEAKKLNDAQAPD

SEQ ID NO: 40 - protein, 58 aa, Artificial Sequence
  SpA6c(Lys4Arg,Lys7Glu,Asn11Lys,Glu15Ala,Asn21Tyr,Gly29Ala,Lys58Va l)
ADNRFNEEQQKAFYAILHLPYLTEEQRNAFIQSLKDDPSVSKEILAEAKKLNDAQAPV